European Patent Application EP 4 803 088 A1, published September 9, 2026. Title: 用于靶向性降解骨硬化蛋白的适体缀合物. Applicant: 安沛治疗有限公司. The sequence listing filed with the application follows.

SEQUENCE LISTING (17 sequences)

SEQ ID NO: 1 - DNA, 42 bp, synthetic construct
  source 1..42: mol_type = other DNA
cccagacgagacacctcatgcttttccccgggggaggggtat

SEQ ID NO: 2 - DNA, 76 bp, synthetic construct
  source 1..76: mol_type = other DNA
cgtacggtcgacgctagctggaagggtgggggcggggggtcctcgcctcgaacgtacgcacgtggagctcggatcc

SEQ ID NO: 3 - DNA, 76 bp, synthetic construct
  source 1..76: mol_type = other DNA
cgtacggtcgacgctagctgggggtagggggaccctggctagttagtcaccgtttcgacacgtggagctcggatcc

SEQ ID NO: 4 - DNA, 76 bp, synthetic construct
  source 1..76: mol_type = other DNA
cgtacggtcgacgctagcgagggggccaactatgcttagtgggggggttgaccgtatccacgtggagctcggatcc

SEQ ID NO: 5 - DNA, 76 bp, synthetic construct
  source 1..76: mol_type = other DNA
cgtacggtcgacgctagcgggtggattaagggggccccgtctgtaggcgattggcgaacacgtggagctcggatcc

SEQ ID NO: 6 - DNA, 76 bp, synthetic construct
  source 1..76: mol_type = other DNA
cgtacggtcgacgctagctgggggtagggggtccttggctacggtgattcggatgtgacacgtggagctcggatcc

SEQ ID NO: 7 - DNA, 56 bp, synthetic construct
  source 1..56: mol_type = other DNA
cgtacggtcgacgctagctcttgttcatcgatcctacgcacgtggagctcggatcc

SEQ ID NO: 8 - DNA, 54 bp, synthetic construct
  source 1..54: mol_type = other DNA
cgtacggtcgacgctagccagccaaagacagagatgcacgtggagctcggatcc

SEQ ID NO: 9 - DNA, 55 bp, synthetic construct
  source 1..55: mol_type = other DNA
cgtacggtcgacgctagctgttgtacatcgccttacgcacgtggagctcggatcc

SEQ ID NO: 10 - DNA, 56 bp, synthetic construct
  source 1..56: mol_type = other DNA
cgtacggtcgacgctagctgttgttcatcgacttgacgcacgtggagctcggatcc

SEQ ID NO: 11 - DNA, 51 bp, synthetic construct
  source 1..51: mol_type = other DNA
cgtacggtcgacgctagccggcgaaattgctaccacgtggagctcggatcc

SEQ ID NO: 12 - DNA, 52 bp, synthetic construct
  source 1..52: mol_type = other DNA
cgtacggtcgacgctagccgttgactcgttgctacacgtggagctcggatcc

SEQ ID NO: 13 - DNA, 55 bp, synthetic construct
  source 1..55: mol_type = other DNA
cgtacggtcgacgctagctggtttcatcgatcgtatccacgtggagctcggatcc

SEQ ID NO: 14 - DNA, 55 bp, synthetic construct
  source 1..55: mol_type = other DNA
cgtacggtcgacgctagctgggtttatcgactagttccacgtggagctcggatcc

SEQ ID NO: 15 - DNA, 51 bp, synthetic construct
  source 1..51: mol_type = other DNA
cgtacggtcgacgctagccggagacctgaggttcacgtggagctcggatcc

SEQ ID NO: 16 - DNA, 56 bp, synthetic construct
  source 1..56: mol_type = other DNA
cgtacggtcgacgctagctgtgttaatcgccgtacctccacgtggagctcggatcc

SEQ ID NO: 17 - DNA, 40 bp, synthetic construct
  source 1..40: mol_type = other DNA
cggggtgtgggttcgtcgttagcttgatttggcagctgcc